European Patent Specification EP 4 288 563 B1, published March 26, 2025. Title: Liquid composition for molecular diagnostics by PCR. Applicant: Bioinova, a.s. The sequence listing filed with the application follows.

SEQUENCE LISTING (2 sequences)

SEQ ID NO: 1 - DNA, 23 bp, artificial
  primer Vanabf
ctgtttgaattgtccggtatccc

SEQ ID NO: 2 - DNA, 23 bp, artificial
  primer Vanabr
gagctttgaatatcgcagcctac